European Patent Specification EP 4 019 532 B1, published August 12, 2026. Title: Peptides promoting hair growth and uses thereof. Applicant: CAREGEN CO., LTD. The sequence listing filed with the application follows.

SEQUENCE LISTING (31 sequences)

SEQ ID NO: 1 - protein, 7 aa, Artificial Sequence
  peptide
TKVFPQD

SEQ ID NO: 2 - DNA, 20 bp, Artificial Sequence
  Lef-1 primer_forward
ccagctattgtaacacctca

SEQ ID NO: 3 - DNA, 20 bp, Artificial Sequence
  Lef-1 primer_reverse
ttcagatgtaggcagctgtc

SEQ ID NO: 4 - DNA, 28 bp, Artificial Sequence
  Cyclin D1 primer_forward
accttcgttgccctctgtgccacagatg

SEQ ID NO: 5 - DNA, 21 bp, Artificial Sequence
  Cyclin D1 primer_reverse
aggcccggaggcagtccgggt

SEQ ID NO: 6 - DNA, 25 bp, Artificial Sequence
  c-Myc primer_forward
accagcagcgactctgaggaggaac

SEQ ID NO: 7 - DNA, 26 bp, Artificial Sequence
  c-Myc primer_reverse
tgaccctcttggcagcaggatagtcc

SEQ ID NO: 8 - DNA, 25 bp, Artificial Sequence
  GAPDH primer_forward
ggtgtgaacggatttggccgtattg

SEQ ID NO: 9 - DNA, 25 bp, Artificial Sequence
  GAPDH primer_reverse
ccgttgaatttgccgtgagtggagt

SEQ ID NO: 10 - DNA, 23 bp, Artificial Sequence
  VEGF primer_forward
atgaactttctgctgtcttgggt

SEQ ID NO: 11 - DNA, 22 bp, Artificial Sequence
  VEGF primer_reverse
tggccttggtgaggtttgatcc

SEQ ID NO: 12 - DNA, 20 bp, Artificial Sequence
  bFGF primer_forward
tgctggtgatgggagttgta

SEQ ID NO: 13 - DNA, 20 bp, Artificial Sequence
  bFGF primer_reverse
cctccaagtagcagccaaag

SEQ ID NO: 14 - DNA, 20 bp, Artificial Sequence
  KGF primer_forward
tctgtcgaacacagtggtac

SEQ ID NO: 15 - DNA, 20 bp, Artificial Sequence
  KGF primer_reverse
gtgtgtccatttagctgatg

SEQ ID NO: 16 - DNA, 20 bp, Artificial Sequence
  HGF primer_forward
caatgcctctggttcccctt

SEQ ID NO: 17 - DNA, 20 bp, Artificial Sequence
  HGF primer_reverse
cccctcgaggatttcgacag

SEQ ID NO: 18 - DNA, 25 bp, Artificial Sequence
  GAPDH primer_forward
ggtgtgaacggatttggccgtattg

SEQ ID NO: 19 - DNA, 25 bp, Artificial Sequence
  GAPDH primer_reverse
ccgttgaatttgccgtgagtggagt

SEQ ID NO: 20 - DNA, 20 bp, Artificial Sequence
  DKK-1 primer_forward
tgatgagtactgcgctagtc

SEQ ID NO: 21 - DNA, 20 bp, Artificial Sequence
  DKK-1 primer_reverse
ctcctatgcttggtacacac

SEQ ID NO: 22 - DNA, 20 bp, Artificial Sequence
  MSX2 primer_forward
cggtcaagtcggaaaattca

SEQ ID NO: 23 - DNA, 19 bp, Artificial Sequence
  MSX2 primer_reverse
gaggagctgggagtggtaa

SEQ ID NO: 24 - DNA, 20 bp, Artificial Sequence
  HA3-II primer_forward
gatcatcgagctgagacgca

SEQ ID NO: 25 - DNA, 20 bp, Artificial Sequence
  HA3-II primer_reverse
ctggccccagggtatctagt

SEQ ID NO: 26 - DNA, 20 bp, Artificial Sequence
  Keratin 5 primer_forward
ccctcaaggatgccaggaac

SEQ ID NO: 27 - DNA, 19 bp, Artificial Sequence
  Keratin 5 primer_reverse
cactgctacctccggcaag

SEQ ID NO: 28 - DNA, 21 bp, Artificial Sequence
  Keratin 14 primer_forward
ccaagacagaggagctgaacc

SEQ ID NO: 29 - DNA, 21 bp, Artificial Sequence
  Keratin 14 primer_reverse
gactgcgatccagaggagacc

SEQ ID NO: 30 - DNA, 20 bp, Artificial Sequence
  Keratin 19 primer_forward
cgcggcgtatccgtgtcctc

SEQ ID NO: 31 - DNA, 24 bp, Artificial Sequence
  Keratin 19 primer_reverse
agcctgttccgtctcaaacttggt